European Patent Application EP 4 474 016 A1, published December 11, 2024. Title: STRATEGIES TO TARGET EXTRACELLULARLY ACCESSIBLE RAS PROTEIN. Applicant: Julius-Maximilians-Universitaet Wuerzburg. The sequence listing filed with the application follows.

SEQUENCE LISTING (119 sequences)

SEQ ID NO: 1 - protein, 189 aa, Homo sapiens [sequence omitted]

SEQ ID NO: 2 - DNA, 570 bp, Homo sapiens
  source 1..570: mol_type = genomic DNA
atgactgaatataaacttgtggtagttggagctggtggcgtaggcaagagtgccttgacgatacagctaattcagaatcattttgtggacgaatatgatccaacaatagaggattcctacaggaagcaagtagtaattgatggagaaacctgtctcttggatattctcgacacagcaggtcaagaggagtacagtgcaatgagggaccagtacatgaggactggggagggctttctttgtgtatttgccataaataatactaaatcatttgaagatattcaccattatagagaacaaattaaaagagttaaggactctgaagatgtacctatggtcctagtaggaaataaatgtgatttgccttctagaacagtagacacaaaacaggctcaggacttagcaagaagttatggaattccttttattgaaacatcagcaaagacaagacagagagtggaggatgctttttatacattggtgagagagatccgacaatacagattgaaaaaaatcagcaaagaagaaaagactcctggctgtgtgaaaattaaaaaatgcattataatgtaa

SEQ ID NO: 3 - protein, 188 aa, Homo sapiens [sequence omitted]

SEQ ID NO: 4 - DNA, 567 bp, Homo sapiens
  source 1..567: mol_type = genomic DNA
atgactgaatataaacttgtggtagttggagctggtggcgtaggcaagagtgccttgacgatacagctaattcagaatcattttgtggacgaatatgatccaacaatagaggattcctacaggaagcaagtagtaattgatggagaaacctgtctcttggatattctcgacacagcaggtcaagaggagtacagtgcaatgagggaccagtacatgaggactggggagggctttctttgtgtatttgccataaataatactaaatcatttgaagatattcaccattatagagaacaaattaaaagagttaaggactctgaagatgtacctatggtcctagtaggaaataaatgtgatttgccttctagaacagtagacacaaaacaggctcaggacttagcaagaagttatggaattccttttattgaaacatcagcaaagacaagacagggtgttgatgatgccttctatacattagttcgagaaattcgaaaacataaagaaaagatgagcaaagatggtaaaaagaagaaaaagaagtcaaagacaaagtgtgtaattatgtaa

SEQ ID NO: 5 - protein, 189 aa, Homo sapiens
MTEYKLVVVGAGGVGKSALTIQLIQNHFVDEYDPTIEDSYRKQVVIDGETCLLDILDTAGQEEYSAMRDQYMRTGEGFLCVFAINNSKSFADINLYREQIKRVKDSDDVPMVLVGNKCDLPTRTVDTKQAHELAKSYGIPFIETSAKTRQGVEDAFYTLVREIRQYRMKKLNSSDDGTQGCMGLPCVVM

SEQ ID NO: 6 - DNA, 570 bp, Homo sapiens
  source 1..570: mol_type = genomic DNA
atgactgagtacaaactggtggtggttggagcaggtggtgttgggaaaagcgcactgacaatccagctaatccagaaccactttgtagatgaatatgatcccaccatagaggattcttacagaaaacaagtggttatagatggtgaaacctgtttgttggacatactggatacagctggacaagaagagtacagtgccatgagagaccaatacatgaggacaggcgaaggcttcctctgtgtatttgccatcaataatagcaagtcatttgcggatattaacctctacagggagcagattaagcgagtaaaagactcggatgatgtacctatggtgctagtgggaaacaagtgtgatttgccaacaaggacagttgatacaaaacaagcccacgaactggccaagagttacgggattccattcattgaaacctcagccaagaccagacagggtgttgaagatgctttttacacactggtaagagaaatacgccagtaccgaatgaaaaaactcaacagcagtgatgatgggactcagggttgtatgggattgccatgtgtggtgatgtaa

SEQ ID NO: 7 - protein, 189 aa, Homo sapiens
MTEYKLVVVGAGGVGKSALTIQLIQNHFVDEYDPTIEDSYRKQVVIDGETCLLDILDTAGQEEYSAMRDQYMRTGEGFLCVFAINNTKSFEDIHQYREQIKRVKDSDDVPMVLVGNKCDLAARTVESRQAQDLARSYGIPYIETSAKTRQGVEDAFYTLVREIRQHKLRKLNPPDESGPGCMSCKCVLS

SEQ ID NO: 8 - DNA, 570 bp, Homo sapiens
  source 1..570: mol_type = genomic DNA
atgacggaatataagctggtggtggtgggcgccggcggtgtgggcaagagtgcgctgaccatccagctgatccagaaccattttgtggacgaatacgaccccactatagaggattcctaccggaagcaggtggtcattgatggggagacgtgcctgttggacatcctggataccgccggccaggaggagtacagcgccatgcgggaccagtacatgcgcaccggggagggcttcctgtgtgtgtttgccatcaacaacaccaagtcttttgaggacatccaccagtacagggagcagatcaaacgggtgaaggactcggatgacgtgcccatggtgctggtggggaacaagtgtgacctggctgcacgcactgtggaatctcggcaggctcaggacctcgcccgaagctacggcatcccctacatcgagacctcggccaagacccggcagggagtggaggatgccttctacacgttggtgcgtgagatccggcagcacaagctgcggaagctgaaccctcctgatgagagtggccccggctgcatgagctgcaagtgtgtgctctcctga

SEQ ID NO: 9 - protein, 170 aa, Homo sapiens
MTEYKLVVVGAGGVGKSALTIQLIQNHFVDEYDPTIEDSYRKQVVIDGETCLLDILDTAGQEEYSAMRDQYMRTGEGFLCVFAINNTKSFEDIHQYREQIKRVKDSDDVPMVLVGNKCDLAARTVESRQAQDLARSYGIPYIETSAKTRQGSRSGSSSSSGTLWDPPGPM

SEQ ID NO: 10 - DNA, 513 bp, Homo sapiens
  source 1..513: mol_type = genomic DNA
atgacggaatataagctggtggtggtgggcgccggcggtgtgggcaagagtgcgctgaccatccagctgatccagaaccattttgtggacgaatacgaccccactatagaggattcctaccggaagcaggtggtcattgatggggagacgtgcctgttggacatcctggataccgccggccaggaggagtacagcgccatgcgggaccagtacatgcgcaccggggagggcttcctgtgtgtgtttgccatcaacaacaccaagtcttttgaggacatccaccagtacagggagcagatcaaacgggtgaaggactcggatgacgtgcccatggtgctggtggggaacaagtgtgacctggctgcacgcactgtggaatctcggcaggctcaggacctcgcccgaagctacggcatcccctacatcgagacctcggccaagacccggcagggcagccgctctggctctagctccagctccgggaccctctgggaccccccgggacccatgtga

SEQ ID NO: 11 - protein, 189 aa, Homo sapiens
MTEYKLVVVGAAGVGKSALTIQLIQNHFVDEYDPTIEDSYRKQVVIDGETCLLDILDTAGQEEYSAMRDQYMRTGEGFLCVFAINNTKSFEDIHQYREQIKRVKDSDDVPMVLVGNKCDLAARTVESRQAQDLARSYGIPYIETSAKTRQGVEDAFYTLVREIRQHKLRKLNPPDESGPGCMSCKCVLS

SEQ ID NO: 12 - protein, 189 aa, Homo sapiens
MTEYKLVVVGACGVGKSALTIQLIQNHFVDEYDPTIEDSYRKQVVIDGETCLLDILDTAGQEEYSAMRDQYMRTGEGFLCVFAINNTKSFEDIHQYREQIKRVKDSDDVPMVLVGNKCDLAARTVESRQAQDLARSYGIPYIETSAKTRQGVEDAFYTLVREIRQHKLRKLNPPDESGPGCMSCKCVLS

SEQ ID NO: 13 - protein, 189 aa, Homo sapiens
MTEYKLVVVGADGVGKSALTIQLIQNHFVDEYDPTIEDSYRKQVVIDGETCLLDILDTAGQEEYSAMRDQYMRTGEGFLCVFAINNTKSFEDIHQYREQIKRVKDSDDVPMVLVGNKCDLAARTVESRQAQDLARSYGIPYIETSAKTRQGVEDAFYTLVREIRQHKLRKLNPPDESGPGCMSCKCVLS

SEQ ID NO: 14 - protein, 189 aa, Homo sapiens
MTEYKLVVVGARGVGKSALTIQLIQNHFVDEYDPTIEDSYRKQVVIDGETCLLDILDTAGQEEYSAMRDQYMRTGEGFLCVFAINNTKSFEDIHQYREQIKRVKDSDDVPMVLVGNKCDLAARTVESRQAQDLARSYGIPYIETSAKTRQGVEDAFYTLVREIRQHKLRKLNPPDESGPGCMSCKCVLS

SEQ ID NO: 15 - protein, 189 aa, Homo sapiens
MTEYKLVVVGASGVGKSALTIQLIQNHFVDEYDPTIEDSYRKQVVIDGETCLLDILDTAGQEEYSAMRDQYMRTGEGFLCVFAINNTKSFEDIHQYREQIKRVKDSDDVPMVLVGNKCDLAARTVESRQAQDLARSYGIPYIETSAKTRQGVEDAFYTLVREIRQHKLRKLNPPDESGPGCMSCKCVLS

SEQ ID NO: 16 - protein, 189 aa, Homo sapiens [sequence omitted]

SEQ ID NO: 17 - protein, 189 aa, Homo sapiens
MTEYKLVVVGAGCVGKSALTIQLIQNHFVDEYDPTIEDSYRKQVVIDGETCLLDILDTAGQEEYSAMRDQYMRTGEGFLCVFAINNTKSFEDIHQYREQIKRVKDSDDVPMVLVGNKCDLAARTVESRQAQDLARSYGIPYIETSAKTRQGVEDAFYTLVREIRQHKLRKLNPPDESGPGCMSCKCVLS

SEQ ID NO: 18 - protein, 189 aa, Homo sapiens [sequence omitted]

SEQ ID NO: 19 - protein, 189 aa, Homo sapiens
MTEYKLVVVGAGRVGKSALTIQLIQNHFVDEYDPTIEDSYRKQVVIDGETCLLDILDTAGQEEYSAMRDQYMRTGEGFLCVFAINNTKSFEDIHQYREQIKRVKDSDDVPMVLVGNKCDLAARTVESRQAQDLARSYGIPYIETSAKTRQGVEDAFYTLVREIRQHKLRKLNPPDESGPGCMSCKCVLS

SEQ ID NO: 20 - protein, 238 aa, Homo sapiens
QVQLQQPGAELVRPGASVKLSCKTSGYSFTSYWMNWVKQRPGQGLEWIGYINPSTGYTEYNQKFKDKATLTADKSSSTAYMQLSSLTSEDSAVYYCARRDYRYFDVWGAGTTVTVSSGGGGSGGGGSGGGGSDIVMTQSPALMSAALGERVTMTCSASSSVSYMHWYQQKSGTSPKRWIYDTSKLASGVPARFSGSGSGTSYSLTISSMEAEDAATYYCQQWSSNPFTFGSGTKLEIK

SEQ ID NO: 21 - protein, 234 aa, Homo sapiens
GSELVRPGASVKLSCKASGYTFTNYWIHWVKQRPGQGLEWIGNVYPGTGTTYYDEKFKSKASLTVDTSSSTAFMQLSSLTSEDSAVYYCTRIDYESLYFGVWGAGTTLTVSSGGGGSGGGGSGGGGSDIQLTQSPASLSASVGETVTITCRASENIYSYLAWYQQKQGKSPQLLVYAATNLADGVPSRFSGSGSGTQYSLKINSLQSEDFGSYYCQHFWGTPFTFGSGTKLEIK

SEQ ID NO: 22 - protein, 246 aa, Homo sapiens
MAQVKLQESGPELVRPGTSVKVSCKASGYAFTNYLIEWIKQRPGQGLEWIGVIHPGNGGTNYNENFKGKATLTADKSSSTAYMQLSSLTSDDSAVYFCASGNDGSYWGQGTTVTVSSGGGGSGGGGSGGGGSDIELTQSPSSLTVTAGEKVTMSCKSSQSLLNSGDQKIYLTWYQQKPGQPPKLLIYWASTRESGVPDRFTGSVSGTDFTLTISSVQAEDLAVYYCQNDYNYPYTFGGGTKLEIKR

SEQ ID NO: 23 - protein, 136 aa, Homo sapiens
KTSNTIRVFLPNKQRTVVNVRNGMSLHDCLMKALKVRGLQPECCAVFRLLHEHKGKKARLDWNTDAASLIGEELQVDFLDHVPLTTHNFARKTFLKLAFCDICQKFLLNGFRCQTCGYKFHEHCSTKVPTMCVDWS

SEQ ID NO: 24 - protein, 240 aa, Homo sapiens
HPIEIARQLTLLESDLYRAVQPSELVGSVWTKEDKEINSPNLLKMIRHTTNLTLWFEKCIVETENLEERVAVVSRIIEILQVFQELNNFNGVLEVVSAMNSSPVYRLDHTFEQIPSRQKKILEEAHELSEDHYKKYLAKLRSINPPCVPFFGIYLTNILKTEEGNPEVLKRHGKELINFSKRRKVAEITGEIQQYQNQPYCLRVESDIKRFFENLNPMGNSMEKEFTDYLFNKSLEIEPR

SEQ ID NO: 25 - protein, 97 aa, Homo sapiens
GSVSSVPTKLEVVAATPTSLLISWDAPAVTVDYYVITYGETGGNSPVQKFEVPGSKSTATISGLKPGVDYTITVYAWGWHGQVYYYMGSPISINYRT

SEQ ID NO: 26 - protein, 92 aa, Homo sapiens
SSVPTKLEVVAATSLLISWDAPAVTVDYYVITYGETGGNSPVQKFEVPGSKSTATISGLKPGVDYTITVYAWGWHGQVYYYMGSPISINYRT

SEQ ID NO: 27 - protein, 240 aa, Homo sapiens
HPIEIARQLTLLESDLYRKVQPSELVGSVWTKEDKEINSPNLLKMIRHTTNLTLWFEKCIVEAENFEERVAVLSRIIEILQVFQDLNNFNGVLEIVSAVNSVSVYRLDHTFEALQERKRKILDEAVELSQDHFKKYLVKLKSINPPCVPFFGIYLTNILKTEEGNNDFLKKKGKDLINFSKRRKVAEITGEIQQYQNQPYCLRIEPDMRRFFENLNPMGSASEKEFTDYLFNKSLEIEPR

SEQ ID NO: 28 - protein, 232 aa, Homo sapiens
EPIELAEHLTFLEHKSFRRISFTDYQSYVIHGCLENNPTLERSIALFNGISKWVQLMVLSKPTPQQRAEVITKFINVAKKLLQLKNFNTLMAVVGGLSHSSISRLKETHSHLSSEVTKNWNEMTELVSSNGNYCNYRKAFADCDGFKIPILGVHLKDLIAVHVIFPDWTEENKVNIVKMHQLSVTLSELVSLQNASHHLEPNMDLINLLTLSLDLYHTEDDIYKLSLVLEPR

SEQ ID NO: 29 - protein, 233 aa, Homo sapiens
SALEIAEQLTLLDHLVFKKIPYEEFFGQGWMKLEKNERTPYIMKTTKHFNDISNLIASEIIRNEDINARVSAIEKWVAVADICRCLHNYNAVLEITSSMNRSAIFRLKKTWLKVSKQTKALIDKLQKLVSSEGRFKNLREALKNCDPPCVPYLGMYLTDLAFIEEGTPNYTEDGLVNFSKMRMISHIIREIRQFQQTAYKIEHQAKVTQYLLDQSFVMDEESLYESSLRIEPK

SEQ ID NO: 30 - protein, 232 aa, Homo sapiens
EPEELSEHLTYLEFKSFRRISFSDYQNYLVNSCVKENPTMERSIALCNGISQWVQLMVLSRPTPQLRAEVFIKFIQVAQKLHQLQNFNTLMAVIGGLCHSSISRLKETSSHVPHEINKVLGEMTELLSSSRNYDNYRRAYGECTDFKIPILGVHLKDLISLYEAMPDYLEDGKVNVHKLLALYNHISELVQLQEVAPPLEANKDLVHLLTLSLDLYYTEDEIYELSYAREPR

SEQ ID NO: 31 - protein, 234 aa, Homo sapiens
EPMELAEHLTYLEYRSFCKILFQDYHSFVTHGCTVDNPVLERFISLFNSVSQWVQLMILSKPTAPQRALVITHFVHVAEKLLQLQNFNTLMAVVGGLSHSSISRLKETHSHVSPETIKLWEGLTELVTATGNYGNYRRRLAACVGFRFPILGVHLKDLVALQLALPDWLDPARTRLNGAKMKQLFSILEELAMVTSLRPPVQANPDLLSLLTVSLDQYQTEDELYQLSLQREPR

SEQ ID NO: 32 - protein, 8 aa, Homo sapiens
HHHHHHHH

SEQ ID NO: 33 - protein, 6 aa, Homo sapiens
HHHHHH

SEQ ID NO: 34 - protein, 17 aa, Homo sapiens
GSGGGGSGGGGSGGGGS

SEQ ID NO: 35 - protein, 5 aa, Homo sapiens
GSGGS

SEQ ID NO: 36-39 - skipped (4 entries)

SEQ ID NO: 40 - protein, 15 aa, Homo sapiens
GGGGSGGGGSGGGGS

SEQ ID NO: 41 - protein, 25 aa, Homo sapiens
SGGGGSGGGGSGGGGSGGGGSGGGG

SEQ ID NO: 42 - protein, 242 aa, Homo sapiens
ASGGGGSGSGGGGGSDKTHTCPPCPAPEAAGGPSVFLFPPKPKDTLMISRTPEVTCVVVDVSHEDPEVKFNWYVDGVEVHNAKTKPREEQYASTYRVVSVLTVLHQDWLNGKEYKCKVSNKALAAPIEKTISKAKGQPREPQVYTLPPCRDELTKNQVSLWCLVKGFYPSDIAVEWESNGQPENNYKTTPPVLDSDGSFFLYSKLTVDKSRWQQGNVFSCSVMHEALHNHYTQKSLSLSPGK

SEQ ID NO: 43 - protein, 229 aa, Homo sapiens
DKTHTCPPCPAPEAAGGPSVFLFPPKPKDTLMISRTPEVTCVVVDVSHEDPEVKFNWYVDGVEVHNAKTKPREEQYASTYRVVSVLTVLHQDWLNGKEYKCKVSNKALAAPIEKTISKAKGQPREPQVCTLPPSRDELTKNQVSLSCAVKGFYPSDIAVEWESNGQPENNYKTTPPVLDSDGSFFLVSKLTVDKSRWQQGNVFSCSVMHEALHNHYTQKSLSLSPGKGS

SEQ ID NO: 44 - protein, 20 aa, Homo sapiens
METDTLLVFVLLVWVPAGNG

SEQ ID NO: 45 - protein, 125 aa, Homo sapiens
EPGEATGEGEPVNNKWLDNAGKDLGSPVPDRIADKLRDQEFESFDDFRETFWEEVSKDPELSKQFSRNNNDRMKVGKAPKTRTQDVSGKRTSFELNHEKPIEENGGVYDMDNISVVTPKRNIDIE

SEQ ID NO: 46 - protein, 130 aa, Homo sapiens
SKSNEPGKATGEGKPVNNKWLNNAGKDLGSPVPDRIANKLRDKEFESFDDFRETFWEEVSKDPELSKQFSRNNNDRMKVGKAPKTRTQDVSGKRTSFELNHQKPIEQNGGVYDMDNISVVTPKRNIDIEG

SEQ ID NO: 47 - protein, 8 aa, Homo sapiens
LEVLFQGP

SEQ ID NO: 48 - protein, 240 aa, Homo sapiens
DVQLVQSGAEVKKPGASVKVSCKASGYTFTRYTMHWVRQAPGQGLEWIGYINPSRGYTNYADSVKGRFTITTDKSTSTAYMELSSLRSEDTATYYCARYYDDHYCLDYWGQGTTVTVSSGGGGSGGGGSGGGGSDIVLTQSPATLSLSPGERATLSCRASQSVSYMNWYQQKPGKAPKRWIYDTSKVASGVPARFSGSGSGTDYSLTINSLEAEDAATYYCQQWSSNPLTFGGGTKVEIK

SEQ ID NO: 49 - protein, 244 aa, Homo sapiens
EVQLVESGGGLVQPGGSLRLSCAASGYSFTGYTMNWVRQAPGKGLEWVALINPYKGVSTYNQKFKDRFTISVDKSKNTAYLQMNSLRAEDTAVYYCARSGYYGDSDWYFDVWGQGTLVTVSSGGGGSGGGGSGGGGSDIQMTQSPSSLSASVGDRVTITCRASQDIRNYLNWYQQKPGKAPKLLIYYTSRLESGVPSRFSGSGSGTDYTLTISSLQPEDFATYYCQQGNTLPWTFGQGTKVEIK

SEQ ID NO: 50 - protein, 7 aa, Homo sapiens
GYTFTRY

SEQ ID NO: 51 - protein, 5 aa, Homo sapiens
NPSRG

SEQ ID NO: 52 - protein, 6 aa, Homo sapiens
YDDHYC

SEQ ID NO: 53 - protein, 7 aa, Homo sapiens
GYSFTGY

SEQ ID NO: 54 - protein, 5 aa, Homo sapiens
NPYKG

SEQ ID NO: 55 - protein, 10 aa, Homo sapiens
SGYYGDSDWY

SEQ ID NO: 56 - protein, 8 aa, Homo sapiens
ASQSVSYM

SEQ ID NO: 57 - protein, 6 aa, Homo sapiens
YDTSKV

SEQ ID NO: 58 - protein, 9 aa, Homo sapiens
QQWSSNPLT

SEQ ID NO: 59 - protein, 9 aa, Homo sapiens
ASQDIRNYL

SEQ ID NO: 60 - protein, 7 aa, Homo sapiens
YTSRLES

SEQ ID NO: 61 - protein, 9 aa, Homo sapiens
QQGNTLPWT

SEQ ID NO: 62 - protein, 119 aa, Homo sapiens
DVQLVQSGAEVKKPGASVKVSCKASGYTFTRYTMHWVRQAPGQGLEWIGYINPSRGYTNYADSVKGRFTITTDKSTSTAYMELSSLRSEDTATYYCARYYDDHYCLDYWGQGTTVTVSS

SEQ ID NO: 63 - protein, 106 aa, Homo sapiens
DIVLTQSPATLSLSPGERATLSCRASQSVSYMNWYQQKPGKAPKRWIYDTSKVASGVPARFSGSGSGTDYSLTINSLEAEDAATYYCQQWSSNPLTFGGGTKVEIK

SEQ ID NO: 64 - protein, 122 aa, Homo sapiens [sequence omitted]

SEQ ID NO: 65 - protein, 107 aa, Homo sapiens [sequence omitted]

SEQ ID NO: 66 - protein, 117 aa, Homo sapiens
QVQLQQPGAELVRPGASVKLSCKTSGYSFTSYWMNWVKQRPGQGLEWIGYINPSTGYTEYNQKFKDKATLTADKSSSTAYMQLSSLTSEDSAVYYCARRDYRYFDVWGAGTTVTVSS

SEQ ID NO: 67 - protein, 106 aa, Homo sapiens
DIVMTQSPALMSAALGERVTMTCSASSSVSYMHWYQQKSGTSPKRWIYDTSKLASGVPARFSGSGSGTSYSLTISSMEAEDAATYYCQQWSSNPFTFGSGTKLEIK

SEQ ID NO: 68 - protein, 112 aa, Homo sapiens
GSELVRPGASVKLSCKASGYTFTNYWIHWVKQRPGQGLEWIGNVYPGTGTTYYDEKFKSKASLTVDTSSSTAFMQLSSLTSEDSAVYYCTRIDYESLYFGVWGAGTTLTVSS

SEQ ID NO: 69 - protein, 107 aa, Homo sapiens
DIQLTQSPASLSASVGETVTITCRASENIYSYLAWYQQKQGKSPQLLVYAATNLADGVPSRFSGSGSGTQYSLKINSLQSEDFGSYYCQHFWGTPFTFGSGTKLEIK

SEQ ID NO: 70 - protein, 117 aa, Homo sapiens
MAQVKLQESGPELVRPGTSVKVSCKASGYAFTNYLIEWIKQRPGQGLEWIGVIHPGNGGTNYNENFKGKATLTADKSSSTAYMQLSSLTSDDSAVYFCASGNDGSYWGQGTTVTVSS

SEQ ID NO: 71 - protein, 114 aa, Homo sapiens
DIELTQSPSSLTVTAGEKVTMSCKSSQSLLNSGDQKIYLTWYQQKPGQPPKLLIYWASTRESGVPDRFTGSVSGTDFTLTISSVQAEDLAVYYCQNDYNYPYTFGGGTKLEIKR

SEQ ID NO: 72 - protein, 226 aa, Homo sapiens
AAATTTPAPRPPTPAPTIASQPLSLRPEACRPAAGGAVHTRGLDFACDIYIWAPLAGTCGVLLLSLVITLYCKRGRKKLLYIFKQPFMRPVQTTQEEDGCSCRFPEEEEGGCELRVKFSRSADAPAYQQGQNQLYNELNLGRREEYDVLDKRRGRDPEMGGKPRRKNPQEGLYNELQKDKMAEAYSEIGMKGERRRGKGHDGLYQGLSTATKDTYDALHMQALPPR

SEQ ID NO: 73 - protein, 479 aa, Homo sapiens
GPGADVQLVQSGAEVKKPGASVKVSCKASGYTFTRYTMHWVRQAPGQGLEWIGYINPSRGYTNYADSVKGRFTITTDKSTSTAYMELSSLRSEDTATYYCARYYDDHYCLDYWGQGTTVTVSSGGGGSGGGGSGGGGSDIVLTQSPATLSLSPGERATLSCRASQSVSYMNWYQQKPGKAPKRWIYDTSKVASGVPARFSGSGSGTDYSLTINSLEAEDAATYYCQQWSSNPLTFGGGTKVEIKGSGGGGGSDKTHTCPPCPAPEAAGGPSVFLFPPKPKDTLMISRTPEVTCVVVDVSHEDPEVKFNWYVDGVEVHNAKTKPREEQYASTYRVVSVLTVLHQDWLNGKEYKCKVSNKALAAPIEKTISKAKGQPREPQVYTLPPCRDELTKNQVSLWCLVKGFYPSDIAVEWESNGQPENNYKTTPPVLDSDGSFFLYSKLTVDKSRWQQGNVFSCSVMHEALHNHYTQKSLSLSPGK

SEQ ID NO: 74 - protein, 480 aa, Homo sapiens
DKTHTCPPCPAPEAAGGPSVFLFPPKPKDTLMISRTPEVTCVVVDVSHEDPEVKFNWYVDGVEVHNAKTKPREEQYASTYRVVSVLTVLHQDWLNGKEYKCKVSNKALAAPIEKTISKAKGQPREPQVCTLPPSRDELTKNQVSLSCAVKGFYPSDIAVEWESNGQPENNYKTTPPVLDSDGSFFLVSKLTVDKSRWQQGNVFSCSVMHEALHNHYTQKSLSLSPGKGSGGSQVQLQQPGAELVRPGASVKLSCKTSGYSFTSYWMNWVKQRPGQGLEWIGYINPSTGYTEYNQKFKDKATLTADKSSSTAYMQLSSLTSEDSAVYYCARRDYRYFDVWGAGTTVTVSSGGGGSGGGGSGGGGSDIVMTQSPALMSAALGERVTMTCSASSSVSYMHWYQQKSGTSPKRWIYDTSKLASGVPARFSGSGSGTSYSLTISSMEAEDAATYYCQQWSSNPFTFGSGTKLEIKGSHHHHHHHH

SEQ ID NO: 75 - protein, 483 aa, Homo sapiens
GPGAEVQLVESGGGLVQPGGSLRLSCAASGYSFTGYTMNWVRQAPGKGLEWVALINPYKGVSTYNQKFKDRFTISVDKSKNTAYLQMNSLRAEDTAVYYCARSGYYGDSDWYFDVWGQGTLVTVSSGGGGSGGGGSGGGGSDIQMTQSPSSLSASVGDRVTITCRASQDIRNYLNWYQQKPGKAPKLLIYYTSRLESGVPSRFSGSGSGTDYTLTISSLQPEDFATYYCQQGNTLPWTFGQGTKVEIKGSGGGGGSDKTHTCPPCPAPEAAGGPSVFLFPPKPKDTLMISRTPEVTCVVVDVSHEDPEVKFNWYVDGVEVHNAKTKPREEQYASTYRVVSVLTVLHQDWLNGKEYKCKVSNKALAAPIEKTISKAKGQPREPQVYTLPPCRDELTKNQVSLWCLVKGFYPSDIAVEWESNGQPENNYKTTPPVLDSDGSFFLYSKLTVDKSRWQQGNVFSCSVMHEALHNHYTQKSLSLSPGK

SEQ ID NO: 76 - protein, 339 aa, Homo sapiens
DKTHTCPPCPAPEAAGGPSVFLFPPKPKDTLMISRTPEVTCVVVDVSHEDPEVKFNWYVDGVEVHNAKTKPREEQYASTYRVVSVLTVLHQDWLNGKEYKCKVSNKALAAPIEKTISKAKGQPREPQVCTLPPSRDELTKNQVSLSCAVKGFYPSDIAVEWESNGQPENNYKTTPPVLDSDGSFFLVSKLTVDKSRWQQGNVFSCSVMHEALHNHYTQKSLSLSPGKGSGGSGSVSSVPTKLEVVAATPTSLLISWDAPAVTVDYYVITYGETGGNSPVQKFEVPGSKSTATISGLKPGVDYTITVYAWGWHGQVYYYMGSPISINYRTGSHHHHHHHH

SEQ ID NO: 77 - protein, 189 aa, Homo sapiens
MTEYKLVVVGAGSVGKSALTIQLIQNHFVDEYDPTIEDSYRKQVVIDGETCLLDILDTAGQEEYSAMRDQYMRTGEGFLCVFAINNTKSFEDIHQYREQIKRVKDSDDVPMVLVGNKCDLAARTVESRQAQDLARSYGIPYIETSAKTRQGVEDAFYTLVREIRQHKLRKLNPPDESGPGCMSCKCVLS

SEQ ID NO: 78 - protein, 189 aa, Homo sapiens
MTEYKLVVVGAGVVGKSALTIQLIQNHFVDEYDPTIEDSYRKQVVIDGETCLLDILDTAGQEEYSAMRDQYMRTGEGFLCVFAINNTKSFEDIHQYREQIKRVKDSDDVPMVLVGNKCDLAARTVESRQAQDLARSYGIPYIETSAKTRQGVEDAFYTLVREIRQHKLRKLNPPDESGPGCMSCKCVLS

SEQ ID NO: 79 - protein, 189 aa, Homo sapiens
MTEYKLVVVGAGGVGKSALTIQLIQNHFVDEYDPTIEDSYRKQVVIDGETCLLDILDTAGHEEYSAMRDQYMRTGEGFLCVFAINNTKSFEDIHQYREQIKRVKDSDDVPMVLVGNKCDLAARTVESRQAQDLARSYGIPYIETSAKTRQGVEDAFYTLVREIRQHKLRKLNPPDESGPGCMSCKCVLS

SEQ ID NO: 80 - protein, 189 aa, Homo sapiens
MTEYKLVVVGAGGVGKSALTIQLIQNHFVDEYDPTIEDSYRKQVVIDGETCLLDILDTAGKEEYSAMRDQYMRTGEGFLCVFAINNTKSFEDIHQYREQIKRVKDSDDVPMVLVGNKCDLAARTVESRQAQDLARSYGIPYIETSAKTRQGVEDAFYTLVREIRQHKLRKLNPPDESGPGCMSCKCVLS

SEQ ID NO: 81 - protein, 189 aa, Homo sapiens
MTEYKLVVVGAGGVGKSALTIQLIQNHFVDEYDPTIEDSYRKQVVIDGETCLLDILDTAGLEEYSAMRDQYMRTGEGFLCVFAINNTKSFEDIHQYREQIKRVKDSDDVPMVLVGNKCDLAARTVESRQAQDLARSYGIPYIETSAKTRQGVEDAFYTLVREIRQHKLRKLNPPDESGPGCMSCKCVLS

SEQ ID NO: 82 - protein, 189 aa, Homo sapiens
MTEYKLVVVGAGGVGKSALTIQLIQNHFVDEYDPTIEDSYRKQVVIDGETCLLDILDTAGPEEYSAMRDQYMRTGEGFLCVFAINNTKSFEDIHQYREQIKRVKDSDDVPMVLVGNKCDLAARTVESRQAQDLARSYGIPYIETSAKTRQGVEDAFYTLVREIRQHKLRKLNPPDESGPGCMSCKCVLS

SEQ ID NO: 83 - protein, 189 aa, Homo sapiens
MTEYKLVVVGAGGVGKSALTIQLIQNHFVDEYDPTIEDSYRKQVVIDGETCLLDILDTAGREEYSAMRDQYMRTGEGFLCVFAINNTKSFEDIHQYREQIKRVKDSDDVPMVLVGNKCDLAARTVESRQAQDLARSYGIPYIETSAKTRQGVEDAFYTLVREIRQHKLRKLNPPDESGPGCMSCKCVLS

SEQ ID NO: 84 - protein, 189 aa, Homo sapiens
MTEYKLVVVGAAGVGKSALTIQLIQNHFVDEYDPTIEDSYRKQVVIDGETCLLDILDTAGQEEYSAMRDQYMRTGEGFLCVFAINNTKSFEDIHHYREQIKRVKDSEDVPMVLVGNKCDLPSRTVDTKQAQDLARSYGIPFIETSAKTRQRVEDAFYTLVREIRQYRLKKISKEEKTPGCVKIKKCIIM

SEQ ID NO: 85 - protein, 189 aa, Homo sapiens
MTEYKLVVVGACGVGKSALTIQLIQNHFVDEYDPTIEDSYRKQVVIDGETCLLDILDTAGQEEYSAMRDQYMRTGEGFLCVFAINNTKSFEDIHHYREQIKRVKDSEDVPMVLVGNKCDLPSRTVDTKQAQDLARSYGIPFIETSAKTRQRVEDAFYTLVREIRQYRLKKISKEEKTPGCVKIKKCIIM

SEQ ID NO: 86 - protein, 189 aa, Homo sapiens
MTEYKLVVVGADGVGKSALTIQLIQNHFVDEYDPTIEDSYRKQVVIDGETCLLDILDTAGQEEYSAMRDQYMRTGEGFLCVFAINNTKSFEDIHHYREQIKRVKDSEDVPMVLVGNKCDLPSRTVDTKQAQDLARSYGIPFIETSAKTRQRVEDAFYTLVREIRQYRLKKISKEEKTPGCVKIKKCIIM

SEQ ID NO: 87 - protein, 189 aa, Homo sapiens
MTEYKLVVVGARGVGKSALTIQLIQNHFVDEYDPTIEDSYRKQVVIDGETCLLDILDTAGQEEYSAMRDQYMRTGEGFLCVFAINNTKSFEDIHHYREQIKRVKDSEDVPMVLVGNKCDLPSRTVDTKQAQDLARSYGIPFIETSAKTRQRVEDAFYTLVREIRQYRLKKISKEEKTPGCVKIKKCIIM

SEQ ID NO: 88 - protein, 189 aa, Homo sapiens
MTEYKLVVVGASGVGKSALTIQLIQNHFVDEYDPTIEDSYRKQVVIDGETCLLDILDTAGQEEYSAMRDQYMRTGEGFLCVFAINNTKSFEDIHHYREQIKRVKDSEDVPMVLVGNKCDLPSRTVDTKQAQDLARSYGIPFIETSAKTRQRVEDAFYTLVREIRQYRLKKISKEEKTPGCVKIKKCIIM

SEQ ID NO: 89 - protein, 189 aa, Homo sapiens
MTEYKLVVVGAVGVGKSALTIQLIQNHFVDEYDPTIEDSYRKQVVIDGETCLLDILDTAGQEEYSAMRDQYMRTGEGFLCVFAINNTKSFEDIHHYREQIKRVKDSEDVPMVLVGNKCDLPSRTVDTKQAQDLARSYGIPFIETSAKTRQRVEDAFYTLVREIRQYRLKKISKEEKTPGCVKIKKCIIM

SEQ ID NO: 90 - protein, 189 aa, Homo sapiens
MTEYKLVVVGAGAVGKSALTIQLIQNHFVDEYDPTIEDSYRKQVVIDGETCLLDILDTAGQEEYSAMRDQYMRTGEGFLCVFAINNTKSFEDIHHYREQIKRVKDSEDVPMVLVGNKCDLPSRTVDTKQAQDLARSYGIPFIETSAKTRQRVEDAFYTLVREIRQYRLKKISKEEKTPGCVKIKKCIIM

SEQ ID NO: 91 - protein, 189 aa, Homo sapiens
MTEYKLVVVGAGCVGKSALTIQLIQNHFVDEYDPTIEDSYRKQVVIDGETCLLDILDTAGQEEYSAMRDQYMRTGEGFLCVFAINNTKSFEDIHHYREQIKRVKDSEDVPMVLVGNKCDLPSRTVDTKQAQDLARSYGIPFIETSAKTRQRVEDAFYTLVREIRQYRLKKISKEEKTPGCVKIKKCIIM

SEQ ID NO: 92 - protein, 189 aa, Homo sapiens
MTEYKLVVVGAGDVGKSALTIQLIQNHFVDEYDPTIEDSYRKQVVIDGETCLLDILDTAGQEEYSAMRDQYMRTGEGFLCVFAINNTKSFEDIHHYREQIKRVKDSEDVPMVLVGNKCDLPSRTVDTKQAQDLARSYGIPFIETSAKTRQRVEDAFYTLVREIRQYRLKKISKEEKTPGCVKIKKCIIM

SEQ ID NO: 93 - protein, 189 aa, Homo sapiens
MTEYKLVVVGAGRVGKSALTIQLIQNHFVDEYDPTIEDSYRKQVVIDGETCLLDILDTAGQEEYSAMRDQYMRTGEGFLCVFAINNTKSFEDIHHYREQIKRVKDSEDVPMVLVGNKCDLPSRTVDTKQAQDLARSYGIPFIETSAKTRQRVEDAFYTLVREIRQYRLKKISKEEKTPGCVKIKKCIIM

SEQ ID NO: 94 - protein, 189 aa, Homo sapiens
MTEYKLVVVGAGSVGKSALTIQLIQNHFVDEYDPTIEDSYRKQVVIDGETCLLDILDTAGQEEYSAMRDQYMRTGEGFLCVFAINNTKSFEDIHHYREQIKRVKDSEDVPMVLVGNKCDLPSRTVDTKQAQDLARSYGIPFIETSAKTRQRVEDAFYTLVREIRQYRLKKISKEEKTPGCVKIKKCIIM

SEQ ID NO: 95 - protein, 189 aa, Homo sapiens
MTEYKLVVVGAGVVGKSALTIQLIQNHFVDEYDPTIEDSYRKQVVIDGETCLLDILDTAGQEEYSAMRDQYMRTGEGFLCVFAINNTKSFEDIHHYREQIKRVKDSEDVPMVLVGNKCDLPSRTVDTKQAQDLARSYGIPFIETSAKTRQRVEDAFYTLVREIRQYRLKKISKEEKTPGCVKIKKCIIM

SEQ ID NO: 96 - protein, 189 aa, Homo sapiens
MTEYKLVVVGAGGVGKSALTIQLIQNHFVDEYDPTIEDSYRKQVVIDGETCLLDILDTAGEEEYSAMRDQYMRTGEGFLCVFAINNTKSFEDIHHYREQIKRVKDSEDVPMVLVGNKCDLPSRTVDTKQAQDLARSYGIPFIETSAKTRQRVEDAFYTLVREIRQYRLKKISKEEKTPGCVKIKKCIIM

SEQ ID NO: 97 - protein, 189 aa, Homo sapiens
MTEYKLVVVGAGGVGKSALTIQLIQNHFVDEYDPTIEDSYRKQVVIDGETCLLDILDTAGHEEYSAMRDQYMRTGEGFLCVFAINNTKSFEDIHHYREQIKRVKDSEDVPMVLVGNKCDLPSRTVDTKQAQDLARSYGIPFIETSAKTRQRVEDAFYTLVREIRQYRLKKISKEEKTPGCVKIKKCIIM

SEQ ID NO: 98 - protein, 189 aa, Homo sapiens
MTEYKLVVVGAGGVGKSALTIQLIQNHFVDEYDPTIEDSYRKQVVIDGETCLLDILDTAGKEEYSAMRDQYMRTGEGFLCVFAINNTKSFEDIHHYREQIKRVKDSEDVPMVLVGNKCDLPSRTVDTKQAQDLARSYGIPFIETSAKTRQRVEDAFYTLVREIRQYRLKKISKEEKTPGCVKIKKCIIM

SEQ ID NO: 99 - protein, 189 aa, Homo sapiens
MTEYKLVVVGAGGVGKSALTIQLIQNHFVDEYDPTIEDSYRKQVVIDGETCLLDILDTAGLEEYSAMRDQYMRTGEGFLCVFAINNTKSFEDIHHYREQIKRVKDSEDVPMVLVGNKCDLPSRTVDTKQAQDLARSYGIPFIETSAKTRQRVEDAFYTLVREIRQYRLKKISKEEKTPGCVKIKKCIIM

SEQ ID NO: 100 - protein, 189 aa, Homo sapiens
MTEYKLVVVGAGGVGKSALTIQLIQNHFVDEYDPTIEDSYRKQVVIDGETCLLDILDTAGPEEYSAMRDQYMRTGEGFLCVFAINNTKSFEDIHHYREQIKRVKDSEDVPMVLVGNKCDLPSRTVDTKQAQDLARSYGIPFIETSAKTRQRVEDAFYTLVREIRQYRLKKISKEEKTPGCVKIKKCIIM

SEQ ID NO: 101 - protein, 189 aa, Homo sapiens
MTEYKLVVVGAGGVGKSALTIQLIQNHFVDEYDPTIEDSYRKQVVIDGETCLLDILDTAGREEYSAMRDQYMRTGEGFLCVFAINNTKSFEDIHHYREQIKRVKDSEDVPMVLVGNKCDLPSRTVDTKQAQDLARSYGIPFIETSAKTRQRVEDAFYTLVREIRQYRLKKISKEEKTPGCVKIKKCIIM

SEQ ID NO: 102 - protein, 189 aa, Homo sapiens
MTEYKLVVVGAAGVGKSALTIQLIQNHFVDEYDPTIEDSYRKQVVIDGETCLLDILDTAGQEEYSAMRDQYMRTGEGFLCVFAINNSKSFADINLYREQIKRVKDSDDVPMVLVGNKCDLPTRTVDTKQAHELAKSYGIPFIETSAKTRQGVEDAFYTLVREIRQYRMKKLNSSDDGTQGCMGLPCVVM

SEQ ID NO: 103 - protein, 189 aa, Homo sapiens
MTEYKLVVVGACGVGKSALTIQLIQNHFVDEYDPTIEDSYRKQVVIDGETCLLDILDTAGQEEYSAMRDQYMRTGEGFLCVFAINNSKSFADINLYREQIKRVKDSDDVPMVLVGNKCDLPTRTVDTKQAHELAKSYGIPFIETSAKTRQGVEDAFYTLVREIRQYRMKKLNSSDDGTQGCMGLPCVVM

SEQ ID NO: 104 - protein, 189 aa, Homo sapiens [sequence omitted]

SEQ ID NO: 105 - protein, 189 aa, Homo sapiens [sequence omitted]

SEQ ID NO: 106 - protein, 189 aa, Homo sapiens
MTEYKLVVVGASGVGKSALTIQLIQNHFVDEYDPTIEDSYRKQVVIDGETCLLDILDTAGQEEYSAMRDQYMRTGEGFLCVFAINNSKSFADINLYREQIKRVKDSDDVPMVLVGNKCDLPTRTVDTKQAHELAKSYGIPFIETSAKTRQGVEDAFYTLVREIRQYRMKKLNSSDDGTQGCMGLPCVVM

SEQ ID NO: 107 - protein, 189 aa, Homo sapiens
MTEYKLVVVGAVGVGKSALTIQLIQNHFVDEYDPTIEDSYRKQVVIDGETCLLDILDTAGQEEYSAMRDQYMRTGEGFLCVFAINNSKSFADINLYREQIKRVKDSDDVPMVLVGNKCDLPTRTVDTKQAHELAKSYGIPFIETSAKTRQGVEDAFYTLVREIRQYRMKKLNSSDDGTQGCMGLPCVVM

SEQ ID NO: 108 - protein, 189 aa, Homo sapiens
MTEYKLVVVGAGAVGKSALTIQLIQNHFVDEYDPTIEDSYRKQVVIDGETCLLDILDTAGQEEYSAMRDQYMRTGEGFLCVFAINNSKSFADINLYREQIKRVKDSDDVPMVLVGNKCDLPTRTVDTKQAHELAKSYGIPFIETSAKTRQGVEDAFYTLVREIRQYRMKKLNSSDDGTQGCMGLPCVVM

SEQ ID NO: 109 - protein, 189 aa, Homo sapiens
MTEYKLVVVGAGCVGKSALTIQLIQNHFVDEYDPTIEDSYRKQVVIDGETCLLDILDTAGQEEYSAMRDQYMRTGEGFLCVFAINNSKSFADINLYREQIKRVKDSDDVPMVLVGNKCDLPTRTVDTKQAHELAKSYGIPFIETSAKTRQGVEDAFYTLVREIRQYRMKKLNSSDDGTQGCMGLPCVVM

SEQ ID NO: 110 - protein, 189 aa, Homo sapiens
MTEYKLVVVGAGDVGKSALTIQLIQNHFVDEYDPTIEDSYRKQVVIDGETCLLDILDTAGQEEYSAMRDQYMRTGEGFLCVFAINNSKSFADINLYREQIKRVKDSDDVPMVLVGNKCDLPTRTVDTKQAHELAKSYGIPFIETSAKTRQGVEDAFYTLVREIRQYRMKKLNSSDDGTQGCMGLPCVVM

SEQ ID NO: 111 - protein, 189 aa, Homo sapiens
MTEYKLVVVGAGRVGKSALTIQLIQNHFVDEYDPTIEDSYRKQVVIDGETCLLDILDTAGQEEYSAMRDQYMRTGEGFLCVFAINNSKSFADINLYREQIKRVKDSDDVPMVLVGNKCDLPTRTVDTKQAHELAKSYGIPFIETSAKTRQGVEDAFYTLVREIRQYRMKKLNSSDDGTQGCMGLPCVVM

SEQ ID NO: 112 - protein, 189 aa, Homo sapiens
MTEYKLVVVGAGSVGKSALTIQLIQNHFVDEYDPTIEDSYRKQVVIDGETCLLDILDTAGQEEYSAMRDQYMRTGEGFLCVFAINNSKSFADINLYREQIKRVKDSDDVPMVLVGNKCDLPTRTVDTKQAHELAKSYGIPFIETSAKTRQGVEDAFYTLVREIRQYRMKKLNSSDDGTQGCMGLPCVVM

SEQ ID NO: 113 - protein, 189 aa, Homo sapiens
MTEYKLVVVGAGVVGKSALTIQLIQNHFVDEYDPTIEDSYRKQVVIDGETCLLDILDTAGQEEYSAMRDQYMRTGEGFLCVFAINNSKSFADINLYREQIKRVKDSDDVPMVLVGNKCDLPTRTVDTKQAHELAKSYGIPFIETSAKTRQGVEDAFYTLVREIRQYRMKKLNSSDDGTQGCMGLPCVVM

SEQ ID NO: 114 - protein, 189 aa, Homo sapiens
MTEYKLVVVGAGGVGKSALTIQLIQNHFVDEYDPTIEDSYRKQVVIDGETCLLDILDTAGEEEYSAMRDQYMRTGEGFLCVFAINNSKSFADINLYREQIKRVKDSDDVPMVLVGNKCDLPTRTVDTKQAHELAKSYGIPFIETSAKTRQGVEDAFYTLVREIRQYRMKKLNSSDDGTQGCMGLPCVVM

SEQ ID NO: 115 - protein, 189 aa, Homo sapiens [sequence omitted]

SEQ ID NO: 116 - protein, 189 aa, Homo sapiens
MTEYKLVVVGAGGVGKSALTIQLIQNHFVDEYDPTIEDSYRKQVVIDGETCLLDILDTAGKEEYSAMRDQYMRTGEGFLCVFAINNSKSFADINLYREQIKRVKDSDDVPMVLVGNKCDLPTRTVDTKQAHELAKSYGIPFIETSAKTRQGVEDAFYTLVREIRQYRMKKLNSSDDGTQGCMGLPCVVM

SEQ ID NO: 117 - protein, 189 aa, Homo sapiens [sequence omitted]

SEQ ID NO: 118 - protein, 189 aa, Homo sapiens
MTEYKLVVVGAGGVGKSALTIQLIQNHFVDEYDPTIEDSYRKQVVIDGETCLLDILDTAGPEEYSAMRDQYMRTGEGFLCVFAINNSKSFADINLYREQIKRVKDSDDVPMVLVGNKCDLPTRTVDTKQAHELAKSYGIPFIETSAKTRQGVEDAFYTLVREIRQYRMKKLNSSDDGTQGCMGLPCVVM

SEQ ID NO: 119 - protein, 189 aa, Homo sapiens
MTEYKLVVVGAGGVGKSALTIQLIQNHFVDEYDPTIEDSYRKQVVIDGETCLLDILDTAGREEYSAMRDQYMRTGEGFLCVFAINNSKSFADINLYREQIKRVKDSDDVPMVLVGNKCDLPTRTVDTKQAHELAKSYGIPFIETSAKTRQGVEDAFYTLVREIRQYRMKKLNSSDDGTQGCMGLPCVVM